European Patent Application EP 4 703 725 A1, published March 4, 2026. Title: Modulators of the mitotic cell cycle in cancer cells and uses thereof for the treatment of cancer. Applicant: Chemotherapeutisches Forschungsinstitut Georg-Speyer-Haus. Application EP. The sequence listing filed with the application follows.

SEQUENCE LISTING (60 sequences)

SEQ ID NO: 1 - DNA, 21 bp, Homo sapiens
  source 1..21: mol_type = other DNA
gctgttgactcgatcgaaacc

SEQ ID NO: 2 - DNA, 21 bp, Homo sapiens
  source 1..21: mol_type = other DNA
gcagatattactgcacaaact

SEQ ID NO: 3 - DNA, 19 bp, Homo sapiens
  source 1..19: mol_type = other DNA
gcttcgcgccgtagtctta

SEQ ID NO: 4 - DNA, 22 bp, Homo sapiens
  source 1..22: mol_type = genomic DNA
tgccgcccaatgtcatagacac

SEQ ID NO: 5 - DNA, 22 bp, Homo sapiens
  source 1..22: mol_type = genomic DNA
agagttcgggcagctccttgat

SEQ ID NO: 6 - DNA, 24 bp, Homo sapiens
  source 1..24: mol_type = genomic DNA
gagtcaacccaagccttagtatcc

SEQ ID NO: 7 - DNA, 22 bp, Homo sapiens
  source 1..22: mol_type = genomic DNA
catgggacaaatgcaactgaag

SEQ ID NO: 8 - DNA, 18 bp, Homo sapiens
  source 1..18: mol_type = genomic DNA
gccactttccaatttcac

SEQ ID NO: 9 - DNA, 18 bp, Homo sapiens
  source 1..18: mol_type = genomic DNA
gagcctcttctcatacac

SEQ ID NO: 10 - DNA, 20 bp, Homo sapiens
  source 1..20: mol_type = genomic DNA
ttggatcctacaccgtgacc

SEQ ID NO: 11 - DNA, 20 bp, Homo sapiens
  source 1..20: mol_type = genomic DNA
tagttctggggcacgatacc

SEQ ID NO: 12 - DNA, 20 bp, Homo sapiens
  source 1..20: mol_type = genomic DNA
gctacctgggtcaggacttg

SEQ ID NO: 13 - DNA, 20 bp, Homo sapiens
  source 1..20: mol_type = genomic DNA
cagagagactgctgctgacg

SEQ ID NO: 14 - DNA, 19 bp, Homo sapiens
  source 1..19: mol_type = genomic DNA
agatcccctggatgcatgc

SEQ ID NO: 15 - DNA, 21 bp, Homo sapiens
  source 1..21: mol_type = genomic DNA
cagtttctgaagagcggagca

SEQ ID NO: 16 - DNA, 21 bp, Homo sapiens
  source 1..21: mol_type = genomic DNA
atgtaccgagactacggggaa

SEQ ID NO: 17 - DNA, 19 bp, Homo sapiens
  source 1..19: mol_type = genomic DNA
ctgctgctgtcgatgcttg

SEQ ID NO: 18 - DNA, 20 bp, Homo sapiens
  source 1..20: mol_type = genomic DNA
acagggcgttttatcttgcg

SEQ ID NO: 19 - DNA, 19 bp, Homo sapiens
  source 1..19: mol_type = genomic DNA
tccaagctcccggctaagt

SEQ ID NO: 20 - DNA, 21 bp, Homo sapiens
  source 1..21: mol_type = genomic DNA
atgtcagctccccaaatgtcc

SEQ ID NO: 21 - DNA, 18 bp, Homo sapiens
  source 1..18: mol_type = genomic DNA
tgcctacagccaccctgg

SEQ ID NO: 22 - DNA, 22 bp, Homo sapiens
  source 1..22: mol_type = genomic DNA
agtgaggagctgcagaagtacg

SEQ ID NO: 23 - DNA, 22 bp, Homo sapiens
  source 1..22: mol_type = genomic DNA
acttggtagttctgtggaggtt

SEQ ID NO: 24 - DNA, 20 bp, Homo sapiens
  source 1..20: mol_type = genomic DNA
ttactgccacggcacagtca

SEQ ID NO: 25 - DNA, 26 bp, Homo sapiens
  source 1..26: mol_type = genomic DNA
agttcctccagatatccaagaagaga

SEQ ID NO: 26 - DNA, 22 bp, Homo sapiens
  source 1..22: mol_type = genomic DNA
agctccaagaaaggacgaacat

SEQ ID NO: 27 - DNA, 22 bp, Homo sapiens
  source 1..22: mol_type = genomic DNA
gccctgtaggtgaggttgatct

SEQ ID NO: 28 - DNA, 20 bp, Homo sapiens
  source 1..20: mol_type = genomic DNA
tggctaggctctgtgctttc

SEQ ID NO: 29 - DNA, 20 bp, Homo sapiens
  source 1..20: mol_type = genomic DNA
cttcaggcaggaaagagggg

SEQ ID NO: 30 - DNA, 22 bp, Homo sapiens
  source 1..22: mol_type = genomic DNA
cacggtcgctgtagaagtaaag

SEQ ID NO: 31 - DNA, 22 bp, Homo sapiens
  source 1..22: mol_type = genomic DNA
tctcctcctcttcgttggaata

SEQ ID NO: 32 - DNA, 22 bp, Homo sapiens
  source 1..22: mol_type = genomic DNA
cttgaaccctgtcgtatgctgg

SEQ ID NO: 33 - DNA, 22 bp, Homo sapiens
  source 1..22: mol_type = genomic DNA
ttggtgcaggaatcagtccagg

SEQ ID NO: 34 - DNA, 24 bp, Homo sapiens
  source 1..24: mol_type = genomic DNA
gaatccggaatctaagaccatcaa

SEQ ID NO: 35 - DNA, 20 bp, Homo sapiens
  source 1..20: mol_type = genomic DNA
gtgcgtggcttcactccagt

SEQ ID NO: 36 - DNA, 22 bp, Homo sapiens
  source 1..22: mol_type = genomic DNA
tgcggactacaagcgaatcacg

SEQ ID NO: 37 - DNA, 22 bp, Homo sapiens
  source 1..22: mol_type = genomic DNA
ctcagcttctggataaccctcg

SEQ ID NO: 38 - DNA, 23 bp, Homo sapiens
  source 1..23: mol_type = genomic DNA
gcctctcattgtcaccgaagaac

SEQ ID NO: 39 - DNA, 22 bp, Homo sapiens
  source 1..22: mol_type = genomic DNA
tggctgacgttggagatcacca

SEQ ID NO: 40 - DNA, 22 bp, Homo sapiens
  source 1..22: mol_type = genomic DNA
gaaccaactctccattgcctgg

SEQ ID NO: 41 - DNA, 22 bp, Homo sapiens
  source 1..22: mol_type = genomic DNA
cgtaagaggagaactgccagct

SEQ ID NO: 42 - DNA, 20 bp, Homo sapiens
  source 1..20: mol_type = genomic DNA
accctttccagtctgggtct

SEQ ID NO: 43 - DNA, 20 bp, Homo sapiens
  source 1..20: mol_type = genomic DNA
tcgctgcagttctgtaccac

SEQ ID NO: 44 - DNA, 23 bp, Homo sapiens
  source 1..23: mol_type = genomic DNA
gctggtgaagcagagagactcag

SEQ ID NO: 45 - DNA, 24 bp, Homo sapiens
  source 1..24: mol_type = genomic DNA
ggtgactttatcttcaggtctgct

SEQ ID NO: 46 - DNA, 21 bp, Homo sapiens
  source 1..21: mol_type = genomic DNA
gtgacgttgacatccgtaaag

SEQ ID NO: 47 - DNA, 19 bp, Homo sapiens
  source 1..19: mol_type = genomic DNA
gccggactcatcgtactcc

SEQ ID NO: 48 - DNA, 22 bp, Homo sapiens
  source 1..22: mol_type = genomic DNA
tgccgcccaatgtcatagacac

SEQ ID NO: 49 - DNA, 22 bp, Homo sapiens
  source 1..22: mol_type = genomic DNA
cagctccttgatgcggtccaaa

SEQ ID NO: 50 - DNA, 24 bp, Homo sapiens
  source 1..24: mol_type = genomic DNA
caaggccaaccgcgagaagatgac

SEQ ID NO: 51 - DNA, 25 bp, Homo sapiens
  source 1..25: mol_type = genomic DNA
gccagaggcgtacagggatagcaca

SEQ ID NO: 52 - RNA, 19 nt, synthetic construct
  source 1..19: mol_type = other RNA
gaaatgggtttggaccgca

SEQ ID NO: 53 - RNA, 19 nt, synthetic construct
  source 1..19: mol_type = other RNA
gctgttgactcgatcgaaa

SEQ ID NO: 54 - RNA, 19 nt, synthetic construct
  source 1..19: mol_type = other RNA
gttcttatgtccttggtga

SEQ ID NO: 55 - RNA, 19 nt, synthetic construct
  source 1..19: mol_type = other RNA
aaccagcacttccgagatt

SEQ ID NO: 56 - RNA, 19 nt, synthetic construct
  source 1..19: mol_type = other RNA
tatgacattgggcggcagc

SEQ ID NO: 57 - RNA, 19 nt, synthetic construct
  source 1..19: mol_type = other RNA
aaggacataagaacttcct

SEQ ID NO: 58 - RNA, 19 nt, synthetic construct
  source 1..19: mol_type = other RNA
tgatggttgaaatactggt

SEQ ID NO: 59 - RNA, 18 nt, synthetic construct
  source 1..18: mol_type = other RNA
atttctatcaccaaggac

SEQ ID NO: 60 - RNA, 19 nt, synthetic construct
  source 1..19: mol_type = other RNA
tcgtcgatgaaatcagtgt